European Patent Application EP 4 368 198 A1, published May 15, 2024. Title: Composition for delivering a protein or a polypeptide to a eukaryotic cell. Applicant: Klinikum der Universität München. Application EP. The sequence listing filed with the application follows.

SEQUENCE LISTING (166 sequences)

SEQ ID NO: 1 - protein, 14 aa, synthetic construct
LHHHKKLLHHHKKL

SEQ ID NO: 2 - protein, 13 aa, synthetic construct
KKKKRRRRRKKKK

SEQ ID NO: 3 - protein, 21 aa, synthetic construct
KLLLLKLLLLKLLLLKLLLLK

SEQ ID NO: 4 - protein, 22 aa, synthetic construct
  SITE 2: note = 6-aminohexanoic acid
  SITE 8: note = 6-aminohexanoic acid
  SITE 16: note = 6-aminohexanoic acid
  SITE 20: note = 6-aminohexanoic acid
RXRRARRXRYQFLIRXRARXRA

SEQ ID NO: 5 - protein, 21 aa, synthetic construct
AGYLLGDLLOOLAAAALOOLL

SEQ ID NO: 6 - protein, 16 aa, synthetic construct
RQIKIWFQNRRMKWKK

SEQ ID NO: 7 - protein, 21 aa, synthetic construct
AGYLLGKLLOOLAAAALOOLL

SEQ ID NO: 8 - protein, 21 aa, synthetic construct
AGYLLGKINLKALAALAKKIL

SEQ ID NO: 9 - protein, 28 aa, synthetic construct
ARLARALARALARHLARALARALRACEA

SEQ ID NO: 10 - protein, 28 aa, synthetic construct
AKLAKALAKALAKHLAKALAKALKACEA

SEQ ID NO: 11 - protein, 21 aa, synthetic construct
AGYLLGELLOOLAAAALOOLL

SEQ ID NO: 12 - protein, 21 aa, synthetic construct
LHHHKKLLHHHKKLLHHHKKL

SEQ ID NO: 13 - protein, 8 aa, synthetic construct
KKRRRRKK

SEQ ID NO: 14 - protein, 12 aa, synthetic construct
KKRRRRRRRRKK

SEQ ID NO: 15 - protein, 13 aa, synthetic construct
KKRRRRRRRRRKK

SEQ ID NO: 16 - protein, 7 aa, synthetic construct
KKKRKKK

SEQ ID NO: 17 - protein, 6 aa, synthetic construct
KRRRRK

SEQ ID NO: 18 - protein, 6 aa, synthetic construct
KKRRKK

SEQ ID NO: 19 - protein, 5 aa, synthetic construct
KKRKK

SEQ ID NO: 20 - protein, 5 aa, synthetic construct
HHHKK

SEQ ID NO: 21 - protein, 16 aa, synthetic construct
KETWWETWWTEWWTEW

SEQ ID NO: 22 - protein, 16 aa, synthetic construct
WETWWTEWKETWWTEW

SEQ ID NO: 23 - protein, 16 aa, synthetic construct
WWETTEWWKETWTEWW

SEQ ID NO: 24 - protein, 15 aa, synthetic construct
ETWWETWWTEWWTEW

SEQ ID NO: 25 - protein, 18 aa, synthetic construct
KETWWETWWTEWWTEWWE

SEQ ID NO: 26 - protein, 5 aa, synthetic construct
KETWW

SEQ ID NO: 27 - protein, 5 aa, synthetic construct
WETWW

SEQ ID NO: 28 - protein, 5 aa, synthetic construct
WWETT

SEQ ID NO: 29 - protein, 6 aa, synthetic construct
VVVVVV

SEQ ID NO: 30 - protein, 12 aa, synthetic construct
GACSERSMNFCG

SEQ ID NO: 31 - protein, 7 aa, synthetic construct
SERSMNF

SEQ ID NO: 32 - protein, 21 aa, synthetic construct
FAEKFKEAVKDYFAKFWDGSG

SEQ ID NO: 33 - protein, 12 aa, synthetic construct
FYPSYHSTPQRP

SEQ ID NO: 34 - protein, 8 aa, synthetic construct
YTYQGKLC

SEQ ID NO: 35 - protein, 14 aa, synthetic construct
GGGGGCYTYQGKLC

SEQ ID NO: 36 - protein, 27 aa, synthetic construct
INNNLQRVRELAVQSANSTNSQSDLDS

SEQ ID NO: 37 - protein, 32 aa, synthetic construct
GSGSGINNNLQRVRELAVQSANSTNSQSDLDS

SEQ ID NO: 38 - protein, 12 aa, synthetic construct
TITHFQFGPTVY

SEQ ID NO: 39 - protein, 17 aa, synthetic construct
GSGSGTITHFQFGPTVY

SEQ ID NO: 40 - protein, 12 aa, synthetic construct
GSGCKSTHPLSC

SEQ ID NO: 41 - protein, 12 aa, synthetic construct
GSGCRGDKGPDC

SEQ ID NO: 42 - protein, 14 aa, synthetic construct
GSGSLDAGQYVLVM

SEQ ID NO: 43 - protein, 19 aa, synthetic construct
KANSSYSGNYPYSILFQKF

SEQ ID NO: 44 - protein, 19 aa, synthetic construct
KIAIVNVSSIFQQLPARET

SEQ ID NO: 45 - protein, 22 aa, synthetic construct
GSGKIAIVNVSSIFQQLPARET

SEQ ID NO: 46 - protein, 11 aa, synthetic construct
FHQLPARSPLP

SEQ ID NO: 47 - protein, 15 aa, synthetic construct
GSGSFHQLPARSPLP

SEQ ID NO: 48 - protein, 7 aa, synthetic construct
VKRKKKP

SEQ ID NO: 49 - protein, 7 aa, synthetic construct
VKRKTKP

SEQ ID NO: 50 - protein, 7 aa, synthetic construct
YGLPHKF

SEQ ID NO: 51 - protein, 12 aa, synthetic construct
GACYGLPHKFCG

SEQ ID NO: 52 - protein, 26 aa, synthetic construct
LHHHKKLLHHHKKLGACSERSMNFCG

SEQ ID NO: 53 - protein, 25 aa, synthetic construct
KKKKRRRRRKKKKGACSERSMNFCG

SEQ ID NO: 54 - protein, 27 aa, synthetic construct
WLHHHKKLLHHHKKLGACSERSMNFCG

SEQ ID NO: 55 - protein, 34 aa, synthetic construct
FAEKFKEAVKDYFAKFWDGSGKKKKRRRRRKKKK

SEQ ID NO: 56 - protein, 25 aa, synthetic construct
KKKKRRRRRKKKKFYPSYHSTPQRP

SEQ ID NO: 57 - protein, 28 aa, synthetic construct
LHHHKKLLHHHKKLGGGGGCYTYQGKLC

SEQ ID NO: 58 - protein, 46 aa, synthetic construct
LHHHKKLLHHHKKLGSGSGINNNLQRVRELAVQSANSTNSQSDLDS

SEQ ID NO: 59 - protein, 31 aa, synthetic construct
LHHHKKLLHHHKKLGSGSGTITHFQFGPTVY

SEQ ID NO: 60 - protein, 26 aa, synthetic construct
LHHHKKLLHHHKKLGSGCKSTHPLSC

SEQ ID NO: 61 - protein, 26 aa, synthetic construct
LHHHKKLLHHHKKLGSGCRGDKGPDC

SEQ ID NO: 62 - protein, 28 aa, synthetic construct
LHHHKKLLHHHKKLGSGSLDAGQYVLVM

SEQ ID NO: 63 - protein, 33 aa, synthetic construct
LHHHKKLLHHHKKLKANSSYSGNYPYSILFQKF

SEQ ID NO: 64 - protein, 36 aa, synthetic construct
LHHHKKLLHHHKKLGSGKIAIVNVSSIFQQLPARET

SEQ ID NO: 65 - protein, 29 aa, synthetic construct
LHHHKKLLHHHKKLGSGSFHQLPARSPLP

SEQ ID NO: 66 - protein, 15 aa, synthetic construct
KKRRRRKKVKRKKKP

SEQ ID NO: 67 - protein, 15 aa, synthetic construct
KKRRRRKKVKRKTKP

SEQ ID NO: 68 - protein, 25 aa, synthetic construct
KKKKRRRRRKKKKGACSERSMNFCG

SEQ ID NO: 69 - protein, 25 aa, synthetic construct
KKKKRRRRRKKKKGACYGLPHKFCG

SEQ ID NO: 70 - protein, 25 aa, synthetic construct
KKRRRRRRRRRKKGACSERSMNFCG

SEQ ID NO: 71 - protein, 24 aa, synthetic construct
KKRRRRRRRRKKGACYGLPHKFCG

SEQ ID NO: 72 - protein, 26 aa, synthetic construct
LHHHKKLLHHHKKLGACSERSMNFCG

SEQ ID NO: 73 - protein, 18 aa, synthetic construct
KRRRRKGACSERSMNFCG

SEQ ID NO: 74 - protein, 42 aa, synthetic construct
KETWWETWWTEWWTEWLHHHKKLLHHHKKLGACSERSMNFCG

SEQ ID NO: 75 - protein, 41 aa, synthetic construct
KETWWETWWTEWWTEWKKKKRRRRRKKKKGACSERSMNFCG

SEQ ID NO: 76 - protein, 36 aa, synthetic construct
KETWWETWWTEWWTEWKKKKRRRRRKKKKVKRKKKP

SEQ ID NO: 77 - protein, 48 aa, synthetic construct
KETWWETWWTEWWTEWKKKKRRRRRKKKKGACSERSMNFCGVKRKKKP

SEQ ID NO: 78 - protein, 41 aa, synthetic construct
KETWWETWWTEWWTEWKKKKRRRRRKKKKGACYGLPHKFCG

SEQ ID NO: 79 - protein, 35 aa, synthetic construct
KETWWETWWTEWWTEWLHHHKKLGACSERSMNFCG

SEQ ID NO: 80 - protein, 49 aa, synthetic construct
KETWWETWWTEWWTEWLHHHKKLLHHHKKLLHHHKKLGACSERSMNFCG

SEQ ID NO: 81 - protein, 37 aa, synthetic construct
KETWWETWWTEWWTEWLHHHKKLLHHHKKLVKRKKKP

SEQ ID NO: 82 - protein, 49 aa, synthetic construct
FAEKFKEAVKDYFAKFWDGSGKKKKRRRRRKKKKETWWETWWTEWWTEW

SEQ ID NO: 83 - protein, 41 aa, synthetic construct
KETWWETWWTEWWTEWKKKKRRRRRKKKKFYPSYHSTPQRP

SEQ ID NO: 84 - protein, 29 aa, synthetic construct
KETWWETWWTEWWTEWKKKKRRRRRKKKK

SEQ ID NO: 85 - protein, 44 aa, synthetic construct
KETWWETWWTEWWTEWLHHHKKLLHHHKKLGGGGGCYTYQGKLC

SEQ ID NO: 86 - protein, 62 aa, synthetic construct
KETWWETWWTEWWTEWLHHHKKLLHHHKKLGSGSGINNNLQRVRELAVQSANSTNSQSDLDS

SEQ ID NO: 87 - protein, 47 aa, synthetic construct
KETWWETWWTEWWTEWLHHHKKLLHHHKKLGSGSGTITHFQFGPTVY

SEQ ID NO: 88 - protein, 42 aa, synthetic construct
KETWWETWWTEWWTEWLHHHKKLLHHHKKLGSGCKSTHPLSC

SEQ ID NO: 89 - protein, 42 aa, synthetic construct
KETWWETWWTEWWTEWLHHHKKLLHHHKKLGSGCRGDKGPDC

SEQ ID NO: 90 - protein, 44 aa, synthetic construct
KETWWETWWTEWWTEWLHHHKKLLHHHKKLGSGSLDAGQYVLVM

SEQ ID NO: 91 - protein, 49 aa, synthetic construct
KETWWETWWTEWWTEWLHHHKKLLHHHKKLKANSSYSGNYPYSILFQKF

SEQ ID NO: 92 - protein, 51 aa, synthetic construct
KETWWETWWTEWWTEWLHHHKKLLHHHKKLGSGIAIVNVSSIFQQLPARET

SEQ ID NO: 93 - protein, 45 aa, synthetic construct
KETWWETWWTEWWTEWLHHHKKLLHHHKKLGSGSFHQLPARSPLP

SEQ ID NO: 94 - protein, 37 aa, synthetic construct
KETWWETWWTEWWTEWKLLLLKLLLLKLLLLKLLLLK

SEQ ID NO: 95 - protein, 38 aa, synthetic construct
  SITE 18: note = 6-aminohexanoic acid
  SITE 24: note = 6-aminohexanoic acid
  SITE 32: note = 6-aminohexanoic acid
  SITE 36: note = 6-aminohexanoic acid
KETWWETWWTEWWTEWRXRRARRXRYQFLIRXRARXRA

SEQ ID NO: 96 - protein, 36 aa, synthetic construct
KETWWETWWTEWWTEWGLFGAIAGFIENGWEGMIDG

SEQ ID NO: 97 - protein, 32 aa, synthetic construct
KETWWETWWTEWWTEWRQIKIWFQNRRMKWKK

SEQ ID NO: 98 - protein, 37 aa, synthetic construct
KETWWETWWTEWWTEWAGYLLGKLLOOLAAAALOOLL

SEQ ID NO: 99 - protein, 37 aa, synthetic construct
KETWWETWWTEWWTEWAGYLLGKINLKALAALAKKIL

SEQ ID NO: 100 - protein, 46 aa, synthetic construct
KETWWETWWTEWWTEWWEARLARALARALARHLARALARALRACEA

SEQ ID NO: 101 - protein, 46 aa, synthetic construct
KETWWETWWTEWWTEWWEAKLAKALAKALAKHLAKALAKALKACEA

SEQ ID NO: 102 - protein, 46 aa, synthetic construct
KETWWETWWTEWWTEWWEAGLAGALAGALAGHLAGALAGALGACEA

SEQ ID NO: 103 - protein, 24 aa, synthetic construct
VVVVVVKRRRRKGACSERSMNFCG

SEQ ID NO: 104 - protein, 13 aa, synthetic construct
DDDDEEEEEDDDD

SEQ ID NO: 105 - protein, 13 aa, synthetic construct
EEEEDDDDDEEEE

SEQ ID NO: 106 - protein, 14 aa, synthetic construct
LDDDEELLDDDEEL

SEQ ID NO: 107 - protein, 14 aa, synthetic construct
LEEEDDLLEEEDDL

SEQ ID NO: 108 - protein, 21 aa, synthetic construct
DLLLLDLLLLDLLLLDLLLLD

SEQ ID NO: 109 - protein, 21 aa, synthetic construct
ELLLLELLLLELLLLELLLLE

SEQ ID NO: 110 - protein, 20 aa, synthetic construct
GLFGAIAGFIENGWEGMIDG

SEQ ID NO: 111 - protein, 22 aa, synthetic construct
  SITE 2: note = 6-amino hexanoic acid
  SITE 8: note = 6-amino hexanoic acid
  SITE 16: note = 6-amino hexanoic acid
  SITE 20: note = 6-amino hexanoic acid
EXDDAEEXDYQFLIEXDAEXDA

SEQ ID NO: 112 - protein, 22 aa, synthetic construct
  SITE 2: note = 6-aminohexanoic acid
  SITE 8: note = 6-aminohexanoic acid
  SITE 16: note = 6-aminohexanoic acid
  SITE 20: note = 6-aminohexanoic acid
DXEEADDXEYQFLIDXEADXEA

SEQ ID NO: 113 - protein, 21 aa, synthetic construct
AGYLLGDINLEALAALADDIL

SEQ ID NO: 114 - protein, 21 aa, synthetic construct
AGYLLGEINLDALAALAEEIL

SEQ ID NO: 115 - protein, 28 aa, synthetic construct
ADLADALADALADELADALADALDACEA

SEQ ID NO: 116 - protein, 28 aa, synthetic construct
AELAEALAEALAEDLAEALAEALEACEA

SEQ ID NO: 117 - protein, 21 aa, synthetic construct
LDEDEDLLEDEDELLDEDEDL

SEQ ID NO: 118 - protein, 19 aa, synthetic construct
LEDELLDDEDEDDLLDEDL

SEQ ID NO: 119 - protein, 8 aa, synthetic construct
DDEEEEDD

SEQ ID NO: 120 - protein, 8 aa, synthetic construct
EEDDDDEE

SEQ ID NO: 121 - protein, 12 aa, synthetic construct
DDEEEEEEEEDD

SEQ ID NO: 122 - protein, 12 aa, synthetic construct
EEDDDDDDDDEE

SEQ ID NO: 123 - protein, 7 aa, synthetic construct
DDDEDDD

SEQ ID NO: 124 - protein, 7 aa, synthetic construct
EEEDEEE

SEQ ID NO: 125 - protein, 6 aa, synthetic construct
DEEEED

SEQ ID NO: 126 - protein, 6 aa, synthetic construct
EDDDDE

SEQ ID NO: 127 - protein, 6 aa, synthetic construct
EEDDEE

SEQ ID NO: 128 - protein, 6 aa, synthetic construct
DDEEEE

SEQ ID NO: 129 - protein, 6 aa, synthetic construct
DEDEDE

SEQ ID NO: 130 - protein, 6 aa, synthetic construct
EDEDED

SEQ ID NO: 131 - protein, 5 aa, synthetic construct
EEDEE

SEQ ID NO: 132 - protein, 5 aa, synthetic construct
DDEDD

SEQ ID NO: 133 - protein, 6 aa, synthetic construct
DEDDED

SEQ ID NO: 134 - protein, 6 aa, synthetic construct
EDEEDE

SEQ ID NO: 135 - protein, 4 aa, synthetic construct
DDDD

SEQ ID NO: 136 - protein, 4 aa, synthetic construct
EEEE

SEQ ID NO: 137 - protein, 6 aa, synthetic construct
HHHHHH

SEQ ID NO: 138 - protein, 8 aa, synthetic construct
DYKDDDDK

SEQ ID NO: 139 - protein, 9 aa, synthetic construct
YPYDVPDYA

SEQ ID NO: 140 - protein, 10 aa, synthetic construct
EQKLISEEDL

SEQ ID NO: 141 - protein, 14 aa, synthetic construct
GKPIPNPLLGLDST

SEQ ID NO: 142 - protein, 15 aa, synthetic construct
GLNDIFEAQKIEWHE

SEQ ID NO: 143 - protein, 8 aa, synthetic construct
WSHPQFEK

SEQ ID NO: 144 - protein, 15 aa, synthetic construct
KETAAAKFERQHMDS

SEQ ID NO: 145 - protein, 13 aa, synthetic construct
GAPVPYPDPLEPR

SEQ ID NO: 146 - protein, 6 aa, synthetic construct
GSGGSG

SEQ ID NO: 147 - protein, 9 aa, synthetic construct
GSGGSGGSG

SEQ ID NO: 148 - protein, 12 aa, synthetic construct
GSGGSGGSGGSG

SEQ ID NO: 149 - protein, 15 aa, synthetic construct
GSGGSGGSGGSGGSG

SEQ ID NO: 150 - protein, 4 aa, synthetic construct
GSGS

SEQ ID NO: 151 - protein, 8 aa, synthetic construct
GSGSGSGS

SEQ ID NO: 152 - protein, 12 aa, synthetic construct
GSGSGSGSGSGS

SEQ ID NO: 153 - protein, 16 aa, synthetic construct
GSGSGSGSGSGSGSGS

SEQ ID NO: 154 - protein, 20 aa, synthetic construct
GSGSGSGSGSGSGSGSGSGS

SEQ ID NO: 155 - protein, 4 aa, synthetic construct
GGGG

SEQ ID NO: 156 - protein, 6 aa, synthetic construct
GGGGGG

SEQ ID NO: 157 - protein, 8 aa, synthetic construct
GGGGGGGG

SEQ ID NO: 158 - protein, 10 aa, synthetic construct
GGGGGGGGGG

SEQ ID NO: 159 - protein, 5 aa, synthetic construct
GGGGS

SEQ ID NO: 160 - protein, 10 aa, synthetic construct
GGGGSGGGGS

SEQ ID NO: 161 - protein, 15 aa, synthetic construct
GGGGSGGGGSGGGGS

SEQ ID NO: 162 - protein, 4 aa, synthetic construct
HHHH

SEQ ID NO: 163 - protein, 8 aa, synthetic construct
HHHHHHHH

SEQ ID NO: 164 - protein, 4 aa, synthetic construct
EAAK

SEQ ID NO: 165 - protein, 8 aa, synthetic construct
EAAKEAAK

SEQ ID NO: 166 - protein, 12 aa, synthetic construct
EAAKEAAKEAAK